European Patent Specification EP 3 607 097 B1, published June 21, 2023. Title: BACILLUS HOST CELLS PRODUCING BETA-GALACTOSIDASES AND LACTASES IN THE ABSENCE OF p-NITROBENZYLESTERASE SIDE ACTIVITY. Applicant: DANISCO. The sequence listing filed with the application follows.

SEQUENCE LISTING (26 sequences)

SEQ ID NO: 1 - DNA, 1470 bp, Bacillus subtilis
atgactcatcaaatagtaacgactcaatacggcaaagtaaaaggcacaacggaaaacggcgtacataagtggaaaggcatcccctatgccaagccgcctgtcggacaatggcgttttaaagcacctgagccgcctgaagtgtgggaagatgtgcttgatgccacagcgtacggctctatttgcccgcagccgtctgatttgctgtcactttcgtatactgagctgccccgccagtccgaggattgcttgtatgtcaatgtatttgcgcctgacaccccaagtaaaaatcttcctgtcatggtgtggattcacggaggcgctttttatctaggagcgggcagtgagccattgtatgacggatcaaaacttgcggcacagggagaagtcattgtcgttacattgaactatcggctggggccgtttggctttttgcacttgtcttcatttaatgaggcgtattctgataaccttgggcttttagaccaagccgccgcgctgaaatgggtgcgagagaatatttcagcgtttggcggtgatcccgataacgtaacagtatttggagaatccgccggcgggatgagcattgccgcgctgcttgctatgcctgcggcaaaaggcctgttccagaaagcaatcatggaaagcggcgcttctcgaacgatgacgaaagaacaagcggcgagcacctcggcagcctttttacaggtccttgggattaacgagggccaactggataaattgcatacggtttctgcggaagatttgctaaaagcggctgatcagcttcggattgcagaaaaagaaaatatctttcagctgttcttccagcccgcccttgatccgaaaacgctgcctgaagaaccagaaaaagcgatcgcagaaggggctgcttccggtattccgctattaattggaacaacccgtgatgaaggatatttatttttcaccccggattcagacgttcattctcaggaaacgcttgatgcagcgctcgagtatttactagggaagccgctggcagagaaagttgccgatttgtatccgcgttctctggaaagccaaattcatatgatgactgatttattattttggcgccctgccgtcgcctatgcatccgcacagtctcattacgcccctgtctggatgtacaggttcgattggcacccgaagaagccgccgtacaataaagcgtttcacgcattagagcttccttttgtctttggaaatctggacggattggaacgaatggcaaaagcggagattacggatgaggtgaaacagctttctcacacgatacaatcagcgtggatcacgttcgccaaaacaggaaacccaagcaccgaagctgtgaattggcctgcgtatcatgaagaaacgagagagacgctgattttagactcagagattacgatcgaaaacgatcccgaatctgaaaaaaggcagaagctattcccttcaaaaggagaataa

SEQ ID NO: 2 - protein, 489 aa, Bacillus subtilis [sequence omitted]

SEQ ID NO: 3 - DNA, 5160 bp, Bifidobacterium bifidum
gcagttgaagatgcaacaagaagcgatagcacaacacaaatgtcatcaacaccggaagttgtttattcatcagcggtcgatagcaaacaaaatcgcacaagcgattttgatgcgaactggaaatttatgctgtcagatagcgttcaagcacaagatccggcatttgatgattcagcatggcaacaagttgatctgccgcatgattatagcatcacacagaaatatagccaaagcaatgaagcagaatcagcatatcttccgggaggcacaggctggtatagaaaaagctttacaattgatagagatctggcaggcaaacgcattgcgattaattttgatggcgtctatatgaatgcaacagtctggtttaatggcgttaaactgggcacacatccgtatggctattcaccgttttcatttgatctgacaggcaatgcaaaatttggcggagaaaacacaattgtcgtcaaagttgaaaatagactgccgtcatcaagatggtattcaggcagcggcatttatagagatgttacactgacagttacagatggcgttcatgttggcaataatggcgtcgcaattaaaacaccgtcactggcaacacaaaatggcggagatgtcacaatgaacctgacaacaaaagtcgcgaatgatacagaagcagcagcgaacattacactgaaacagacagtttttccgaaaggcggaaaaacggatgcagcaattggcacagttacaacagcatcaaaatcaattgcagcaggcgcatcagcagatgttacaagcacaattacagcagcaagcccgaaactgtggtcaattaaaaacccgaacctgtatacagttagaacagaagttctgaacggaggcaaagttctggatacatatgatacagaatatggctttcgctggacaggctttgatgcaacatcaggcttttcactgaatggcgaaaaagtcaaactgaaaggcgttagcatgcatcatgatcaaggctcacttggcgcagttgcaaatagacgcgcaattgaaagacaagtcgaaatcctgcaaaaaatgggcgtcaatagcattcgcacaacacataatccggcagcaaaagcactgattgatgtctgcaatgaaaaaggcgttctggttgtcgaagaagtctttgatatgtggaaccgcagcaaaaatggcaacacggaagattatggcaaatggtttggccaagcaattgcaggcgataatgcagttctgggaggcgataaagatgaaacatgggcgaaatttgatcttacatcaacaattaaccgcgatagaaatgcaccgtcagttattatgtggtcactgggcaatgaaatgatggaaggcatttcaggctcagtttcaggctttccggcaacatcagcaaaactggttgcatggacaaaagcagcagattcaacaagaccgatgacatatggcgataacaaaattaaagcgaactggaacgaatcaaatacaatgggcgataatctgacagcaaatggcggagttgttggcacaaattattcagatggcgcaaactatgataaaattcgtacaacacatccgtcatgggcaatttatggctcagaaacagcatcagcgattaatagccgtggcatttataatagaacaacaggcggagcacaatcatcagataaacagctgacaagctatgataattcagcagttggctggggagcagttgcatcatcagcatggtatgatgttgttcagagagattttgtcgcaggcacatatgtttggacaggatttgattatctgggcgaaccgacaccgtggaatggcacaggctcaggcgcagttggctcatggccgtcaccgaaaaatagctattttggcatcgttgatacagcaggctttccgaaagatacatattatttttatcagagccagtggaatgatgatgttcatacactgcatattcttccggcatggaatgaaaatgttgttgcaaaaggctcaggcaataatgttccggttgtcgtttatacagatgcagcgaaagtgaaactgtattttacaccgaaaggctcaacagaaaaaagactgatcggcgaaaaatcatttacaaaaaaaacaacagcggcaggctatacatatcaagtctatgaaggcagcgataaagattcaacagcgcataaaaacatgtatctgacatggaatgttccgtgggcagaaggcacaatttcagcggaagcgtatgatgaaaataatcgcctgattccggaaggcagcacagaaggcaacgcatcagttacaacaacaggcaaagcagcaaaactgaaagcagatgcggatcgcaaaacaattacagcggatggcaaagatctgtcatatattgaagtcgatgtcacagatgcaaatggccatattgttccggatgcagcaaatagagtcacatttgatgttaaaggcgcaggcaaactggttggcgttgataatggctcatcaccggatcatgattcatatcaagcggataaccgcaaagcattttcaggcaaagtcctggcaattgttcagtcaacaaaagaagcaggcgaaattacagttacagcaaaagcagatggcctgcaatcaagcacagttaaaattgcaacaacagcagttccgggaacaagcacagaaaaaacagtccgcagcttttattacagccgcaactattatgtcaaaacaggcaacaaaccgattctgccgtcagatgttgaagttcgctattcagatggaacaagcgatagacaaaacgttacatgggatgcagtttcagatgatcaaattgcaaaagcaggctcattttcagttgcaggcacagttgcaggccaaaaaattagcgttcgcgtcacaatgattgatgaaattggcgcactgctgaattattcagcaagcacaccggttggcacaccggcagttcttccgggatcaagaccggcagtcctgccggatggcacagtcacatcagcaaattttgcagtccattggacaaaaccggcagatacagtctataatacagcaggcacagtcaaagtaccgggaacagcaacagtttttggcaaagaatttaaagtcacagcgacaattagagttcaaagaagccaagttacaattggctcatcagtttcaggaaatgcactgagactgacacaaaatattccggcagataaacaatcagatacactggatgcgattaaagatggctcaacaacagttgatgcaaatacaggcggaggcgcaaatccgtcagcatggacaaattgggcatattcaaaagcaggccataacacagcggaaattacatttgaatatgcgacagaacaacaactgggccagatcgtcatgtatttttttcgcgatagcaatgcagttagatttccggatgctggcaaaacaaaaattcagatcagcgcagatggcaaaaattggacagatctggcagcaacagaaacaattgcagcgcaagaatcaagcgatagagtcaaaccgtatacatatgattttgcaccggttggcgcaacatttgttaaagtgacagtcacaaacgcagatacaacaacaccgtcaggcgttgtttgcgcaggcctgacagaaattgaactgaaaacagcgacaagcaaatttgtcacaaatacatcagcagcactgtcatcacttacagtcaatggcacaaaagtttcagattcagttctggcagcaggctcatataacacaccggcaattatcgcagatgttaaagcggaaggcgaaggcaatgcaagcgttacagtccttccggcacatgataatgttattcgcgtcattacagaaagcgaagatcatgtcacacgcaaaacatttacaatcaacctgggcacagaacaagaatttccggctgattcagatgaaagagattatccggcagcagatatgacagtcacagttggctcagaacaaacatcaggcacagcaacagaaggaccgaaaaaatttgcagtcgatggcaacacatcaacatattggcatagcaattggacaccgacaacagttaatgatctgtggatcgcgtttgaactgcaaaaaccgacaaaactggatgcactgagatatcttccgcgtccggcaggctcaaaaaatggcagcgtcacagaatataaagttcaggtgtcagatgatggaacaaactggacagatgcaggctcaggcacatggacaacggattatggctggaaactggcggaatttaatcaaccggtcacaacaaaacatgttagactgaaagcggttcatacatatgcagatagcggcaacgataaatttatgagcgcaagcgaaattagactgagaaaagcggtcgatacaacggatatttcaggcgcaacagttacagttccggcaaaactgacagttgatagagttgatgcagatcatccggcaacatttgcaacaaaagatgtcacagttacactgggagatgcaacactgagatatggcgttgattatctgctggattatgcaggcaatacagcagttggcaaagcaacagtgacagttagaggcattgataaatattcaggcacagtcgcgaaaacatttacaattgaactgaaaaatgcaccggcaccggaaccgacactgacatcagttagcgtcaaaacaaaaccgagcaaactgacatatgttgtcggagatgcatttgatccggcaggcctggttctgcaacatgatagacaagcagatagacctccgcaaccgctggttggcgaacaagcggatgaacgcggactgacatgcggcacaagatgcgatagagttgaacaactgcgcaaacatgaaaatagagaagcgcatagaacaggcctggatcatctggaatttgttggcgcagcagatggcgcagttggagaacaagcaacatttaaagtccatgtccatgcagatcagggagatggcagacatgatgatgcagatgaacgcgatattgatccgcatgttccggtcgatcatgcagttggcgaactggcaagagcagcatgccatcatgttattggcctgagagtcgatacacatagacttaaagcaagcggctttcaaattccggctgatgatatggcagaaatcgatcgcattacaggctttcatcgttttgaacgccatgtc

SEQ ID NO: 4 - protein, 1720 aa, Bifidobacterium bifidum
VEDATRSDSTTQMSSTPEVVYSSAVDSKQNRTSDFDANWKFMLSDSVQAQDPAFDDSAWQQVDLPHDYSITQKYSQSNEAESAYLPGGTGWYRKSFTIDRDLAGKRIAINFDGVYMNATVWFNGVKLGTHPYGYSPFSFDLTGNAKFGGENTIVVKVENRLPSSRWYSGSGIYRDVTLTVTDGVHVGNNGVAIKTPSLATQNGGDVTMNLTTKVANDTEAAANITLKQTVFPKGGKTDAAIGTVTTASKSIAAGASADVTSTITAASPKLWSIKNPNLYTVRTEVLNGGKVLDTYDTEYGFRWTGFDATSGFSLNGEKVKLKGVSMHHDQGSLGAVANRRAIERQVEILQKMGVNSIRTTHNPAAKALIDVCNEKGVLVVEEVFDMWNRSKNGNTEDYGKWFGQAIAGDNAVLGGDKDETWAKFDLTSTINRDRNAPSVIMWSLGNEMMEGISGSVSGFPATSAKLVAWTKAADSTRPMTYGDNKIKANWNESNTMGDNLTANGGVVGTNYSDGANYDKIRTTHPSWAIYGSETASAINSRGIYNRTTGGAQSSDKQLTSYDNSAVGWGAVASSAWYDVVQRDFVAGTYVWTGFDYLGEPTPWNGTGSGAVGSWPSPKNSYFGIVDTAGFPKDTYYFYQSQWNDDVHTLHILPAWNENVVAKGSGNNVPVVVYTDAAKVKLYFTPKGSTEKRLIGEKSFTKKTTAAGYTYQVYEGSDKDSTAHKNMYLTWNVPWAEGTISAEAYDENNRLIPEGSTEGNASVTTTGKAAKLKADADRKTITADGKDLSYIEVDVTDANGHIVPDAANRVTFDVKGAGKLVGVDNGSSPDHDSYQADNRKAFSGKVLAIVQSTKEAGEITVTAKADGLQSSTVKIATTAVPGTSTEKTVRSFYYSRNYYVKTGNKPILPSDVEVRYSDGTSDRQNVTWDAVSDDQIAKAGSFSVAGTVAGQKISVRVTMIDEIGALLNYSASTPVGTPAVLPGSRPAVLPDGTVTSANFAVHWTKPADTVYNTAGTVKVPGTATVFGKEFKVTATIRVQRSQVTIGSSVSGNALRLTQNIPADKQSDTLDAIKDGSTTVDANTGGGANPSAWTNWAYSKAGHNTAEITFEYATEQQLGQIVMYFFRDSNAVRFPDAGKTKIQISADGKNWTDLAATETIAAQESSDRVKPYTYDFAPVGATFVKVTVTNADTTTPSGVVCAGLTEIELKTATSKFVTNTSAALSSLTVNGTKVSDSVLAAGSYNTPAIIADVKAEGEGNASVTVLPAHDNVIRVITESEDHVTRKTFTINLGTEQEFPADSDERDYPAADMTVTVGSEQTSGTATEGPKKFAVDGNTSTYWHSNWTPTTVNDLWIAFELQKPTKLDALRYLPRPAGSKNGSVTEYKVQVSDDGTNWTDAGSGTWTTDYGWKLAEFNQPVTTKHVRLKAVHTYADSGNDKFMSASEIRLRKAVDTTDISGATVTVPAKLTVDRVDADHPATFATKDVTVTLGDATLRYGVDYLLDYAGNTAVGKATVTVRGIDKYSGTVAKTFTIELKNAPAPEPTLTSVSVKTKPSKLTYVVGDAFDPAGLVLQHDRQADRPPQPLVGEQADERGLTCGTRCDRVEQLRKHENREAHRTGLDHLEFVGAADGAVGEQATFKVHVHADQGDGRHDDADERDIDPHVPVDHAVGELARAACHHVIGLRVDTHRLKASGFQIPADDMAEIDRITGFHRFERHVG

SEQ ID NO: 5 - DNA, 2661 bp, Bifidobacterium bifidum
gttgaagatgcaacaagaagcgatagcacaacacaaatgtcatcaacaccggaagttgtttattcatcagcggtcgatagcaaacaaaatcgcacaagcgattttgatgcgaactggaaatttatgctgtcagatagcgttcaagcacaagatccggcatttgatgattcagcatggcaacaagttgatctgccgcatgattatagcatcacacagaaatatagccaaagcaatgaagcagaatcagcatatcttccgggaggcacaggctggtatagaaaaagctttacaattgatagagatctggcaggcaaacgcattgcgattaattttgatggcgtctatatgaatgcaacagtctggtttaatggcgttaaactgggcacacatccgtatggctattcaccgttttcatttgatctgacaggcaatgcaaaatttggcggagaaaacacaattgtcgtcaaagttgaaaatagactgccgtcatcaagatggtattcaggcagcggcatttatagagatgttacactgacagttacagatggcgttcatgttggcaataatggcgtcgcaattaaaacaccgtcactggcaacacaaaatggcggagatgtcacaatgaacctgacaacaaaagtcgcgaatgatacagaagcagcagcgaacattacactgaaacagacagtttttccgaaaggcggaaaaacggatgcagcaattggcacagttacaacagcatcaaaatcaattgcagcaggcgcatcagcagatgttacaagcacaattacagcagcaagcccgaaactgtggtcaattaaaaacccgaacctgtatacagttagaacagaagttctgaacggaggcaaagttctggatacatatgatacagaatatggctttcgctggacaggctttgatgcaacatcaggcttttcactgaatggcgaaaaagtcaaactgaaaggcgttagcatgcatcatgatcaaggctcacttggcgcagttgcaaatagacgcgcaattgaaagacaagtcgaaatcctgcaaaaaatgggcgtcaatagcattcgcacaacacataatccggcagcaaaagcactgattgatgtctgcaatgaaaaaggcgttctggttgtcgaagaagtctttgatatgtggaaccgcagcaaaaatggcaacacggaagattatggcaaatggtttggccaagcaattgcaggcgataatgcagttctgggaggcgataaagatgaaacatgggcgaaatttgatcttacatcaacaattaaccgcgatagaaatgcaccgtcagttattatgtggtcactgggcaatgaaatgatggaaggcatttcaggctcagtttcaggctttccggcaacatcagcaaaactggttgcatggacaaaagcagcagattcaacaagaccgatgacatatggcgataacaaaattaaagcgaactggaacgaatcaaatacaatgggcgataatctgacagcaaatggcggagttgttggcacaaattattcagatggcgcaaactatgataaaattcgtacaacacatccgtcatgggcaatttatggctcagaaacagcatcagcgattaatagccgtggcatttataatagaacaacaggcggagcacaatcatcagataaacagctgacaagctatgataattcagcagttggctggggagcagttgcatcatcagcatggtatgatgttgttcagagagattttgtcgcaggcacatatgtttggacaggatttgattatctgggcgaaccgacaccgtggaatggcacaggctcaggcgcagttggctcatggccgtcaccgaaaaatagctattttggcatcgttgatacagcaggctttccgaaagatacatattatttttatcagagccagtggaatgatgatgttcatacactgcatattcttccggcatggaatgaaaatgttgttgcaaaaggctcaggcaataatgttccggttgtcgtttatacagatgcagcgaaagtgaaactgtattttacaccgaaaggctcaacagaaaaaagactgatcggcgaaaaatcatttacaaaaaaaacaacagcggcaggctatacatatcaagtctatgaaggcagcgataaagattcaacagcgcataaaaacatgtatctgacatggaatgttccgtgggcagaaggcacaatttcagcggaagcgtatgatgaaaataatcgcctgattccggaaggcagcacagaaggcaacgcatcagttacaacaacaggcaaagcagcaaaactgaaagcagatgcggatcgcaaaacaattacagcggatggcaaagatctgtcatatattgaagtcgatgtcacagatgcaaatggccatattgttccggatgcagcaaatagagtcacatttgatgttaaaggcgcaggcaaactggttggcgttgataatggctcatcaccggatcatgattcatatcaagcggataaccgcaaagcattttcaggcaaagtcctggcaattgttcagtcaacaaaagaagcaggcgaaattacagttacagcaaaagcagatggcctgcaatcaagcacagttaaaattgcaacaacagcagttccgggaacaagcacagaaaaaaca

SEQ ID NO: 6 - protein, 887 aa, Bifidobacterium bifidum
VEDATRSDSTTQMSSTPEVVYSSAVDSKQNRTSDFDANWKFMLSDSVQAQDPAFDDSAWQQVDLPHDYSITQKYSQSNEAESAYLPGGTGWYRKSFTIDRDLAGKRIAINFDGVYMNATVWFNGVKLGTHPYGYSPFSFDLTGNAKFGGENTIVVKVENRLPSSRWYSGSGIYRDVTLTVTDGVHVGNNGVAIKTPSLATQNGGDVTMNLTTKVANDTEAAANITLKQTVFPKGGKTDAAIGTVTTASKSIAAGASADVTSTITAASPKLWSIKNPNLYTVRTEVLNGGKVLDTYDTEYGFRWTGFDATSGFSLNGEKVKLKGVSMHHDQGSLGAVANRRAIERQVEILQKMGVNSIRTTHNPAAKALIDVCNEKGVLVVEEVFDMWNRSKNGNTEDYGKWFGQAIAGDNAVLGGDKDETWAKFDLTSTINRDRNAPSVIMWSLGNEMMEGISGSVSGFPATSAKLVAWTKAADSTRPMTYGDNKIKANWNESNTMGDNLTANGGVVGTNYSDGANYDKIRTTHPSWAIYGSETASAINSRGIYNRTTGGAQSSDKQLTSYDNSAVGWGAVASSAWYDVVQRDFVAGTYVWTGFDYLGEPTPWNGTGSGAVGSWPSPKNSYFGIVDTAGFPKDTYYFYQSQWNDDVHTLHILPAWNENVVAKGSGNNVPVVVYTDAAKVKLYFTPKGSTEKRLIGEKSFTKKTTAAGYTYQVYEGSDKDSTAHKNMYLTWNVPWAEGTISAEAYDENNRLIPEGSTEGNASVTTTGKAAKLKADADRKTITADGKDLSYIEVDVTDANGHIVPDAANRVTFDVKGAGKLVGVDNGSSPDHDSYQADNRKAFSGKVLAIVQSTKEAGEITVTAKADGLQSSTVKIATTAVPGTSTEKT

SEQ ID NO: 7 - DNA, 2895 bp, Bifidobacterium bifidum
gttgaagatgcaacaagaagcgatagcacaacacaaatgtcatcaacaccggaagttgtttattcatcagcggtcgatagcaaacaaaatcgcacaagcgattttgatgcgaactggaaatttatgctgtcagatagcgttcaagcacaagatccggcatttgatgattcagcatggcaacaagttgatctgccgcatgattatagcatcacacagaaatatagccaaagcaatgaagcagaatcagcatatcttccgggaggcacaggctggtatagaaaaagctttacaattgatagagatctggcaggcaaacgcattgcgattaattttgatggcgtctatatgaatgcaacagtctggtttaatggcgttaaactgggcacacatccgtatggctattcaccgttttcatttgatctgacaggcaatgcaaaatttggcggagaaaacacaattgtcgtcaaagttgaaaatagactgccgtcatcaagatggtattcaggcagcggcatttatagagatgttacactgacagttacagatggcgttcatgttggcaataatggcgtcgcaattaaaacaccgtcactggcaacacaaaatggcggagatgtcacaatgaacctgacaacaaaagtcgcgaatgatacagaagcagcagcgaacattacactgaaacagacagtttttccgaaaggcggaaaaacggatgcagcaattggcacagttacaacagcatcaaaatcaattgcagcaggcgcatcagcagatgttacaagcacaattacagcagcaagcccgaaactgtggtcaattaaaaacccgaacctgtatacagttagaacagaagttctgaacggaggcaaagttctggatacatatgatacagaatatggctttcgctggacaggctttgatgcaacatcaggcttttcactgaatggcgaaaaagtcaaactgaaaggcgttagcatgcatcatgatcaaggctcacttggcgcagttgcaaatagacgcgcaattgaaagacaagtcgaaatcctgcaaaaaatgggcgtcaatagcattcgcacaacacataatccggcagcaaaagcactgattgatgtctgcaatgaaaaaggcgttctggttgtcgaagaagtctttgatatgtggaaccgcagcaaaaatggcaacacggaagattatggcaaatggtttggccaagcaattgcaggcgataatgcagttctgggaggcgataaagatgaaacatgggcgaaatttgatcttacatcaacaattaaccgcgatagaaatgcaccgtcagttattatgtggtcactgggcaatgaaatgatggaaggcatttcaggctcagtttcaggctttccggcaacatcagcaaaactggttgcatggacaaaagcagcagattcaacaagaccgatgacatatggcgataacaaaattaaagcgaactggaacgaatcaaatacaatgggcgataatctgacagcaaatggcggagttgttggcacaaattattcagatggcgcaaactatgataaaattcgtacaacacatccgtcatgggcaatttatggctcagaaacagcatcagcgattaatagccgtggcatttataatagaacaacaggcggagcacaatcatcagataaacagctgacaagctatgataattcagcagttggctggggagcagttgcatcatcagcatggtatgatgttgttcagagagattttgtcgcaggcacatatgtttggacaggatttgattatctgggcgaaccgacaccgtggaatggcacaggctcaggcgcagttggctcatggccgtcaccgaaaaatagctattttggcatcgttgatacagcaggctttccgaaagatacatattatttttatcagagccagtggaatgatgatgttcatacactgcatattcttccggcatggaatgaaaatgttgttgcaaaaggctcaggcaataatgttccggttgtcgtttatacagatgcagcgaaagtgaaactgtattttacaccgaaaggctcaacagaaaaaagactgatcggcgaaaaatcatttacaaaaaaaacaacagcggcaggctatacatatcaagtctatgaaggcagcgataaagattcaacagcgcataaaaacatgtatctgacatggaatgttccgtgggcagaaggcacaatttcagcggaagcgtatgatgaaaataatcgcctgattccggaaggcagcacagaaggcaacgcatcagttacaacaacaggcaaagcagcaaaactgaaagcagatgcggatcgcaaaacaattacagcggatggcaaagatctgtcatatattgaagtcgatgtcacagatgcaaatggccatattgttccggatgcagcaaatagagtcacatttgatgttaaaggcgcaggcaaactggttggcgttgataatggctcatcaccggatcatgattcatatcaagcggataaccgcaaagcattttcaggcaaagtcctggcaattgttcagtcaacaaaagaagcaggcgaaattacagttacagcaaaagcagatggcctgcaatcaagcacagttaaaattgcaacaacagcagttccgggaacaagcacagaaaaaacagtccgcagcttttattacagccgcaactattatgtcaaaacaggcaacaaaccgattctgccgtcagatgttgaagttcgctattcagatggaacaagcgatagacaaaacgttacatgggatgcagtttcagatgatcaaattgcaaaagcaggctcattttcagttgcaggcacagttgcaggccaaaaaattagcgttcgcgtcacaatgattgatgaaattggcgcactg

SEQ ID NO: 8 - protein, 965 aa, Bifidobacterium bifidum
VEDATRSDSTTQMSSTPEVVYSSAVDSKQNRTSDFDANWKFMLSDSVQAQDPAFDDSAWQQVDLPHDYSITQKYSQSNEAESAYLPGGTGWYRKSFTIDRDLAGKRIAINFDGVYMNATVWFNGVKLGTHPYGYSPFSFDLTGNAKFGGENTIVVKVENRLPSSRWYSGSGIYRDVTLTVTDGVHVGNNGVAIKTPSLATQNGGDVTMNLTTKVANDTEAAANITLKQTVFPKGGKTDAAIGTVTTASKSIAAGASADVTSTITAASPKLWSIKNPNLYTVRTEVLNGGKVLDTYDTEYGFRWTGFDATSGFSLNGEKVKLKGVSMHHDQGSLGAVANRRAIERQVEILQKMGVNSIRTTHNPAAKALIDVCNEKGVLVVEEVFDMWNRSKNGNTEDYGKWFGQAIAGDNAVLGGDKDETWAKFDLTSTINRDRNAPSVIMWSLGNEMMEGISGSVSGFPATSAKLVAWTKAADSTRPMTYGDNKIKANWNESNTMGDNLTANGGVVGTNYSDGANYDKIRTTHPSWAIYGSETASAINSRGIYNRTTGGAQSSDKQLTSYDNSAVGWGAVASSAWYDVVQRDFVAGTYVWTGFDYLGEPTPWNGTGSGAVGSWPSPKNSYFGIVDTAGFPKDTYYFYQSQWNDDVHTLHILPAWNENVVAKGSGNNVPVVVYTDAAKVKLYFTPKGSTEKRLIGEKSFTKKTTAAGYTYQVYEGSDKDSTAHKNMYLTWNVPWAEGTISAEAYDENNRLIPEGSTEGNASVTTTGKAAKLKADADRKTITADGKDLSYIEVDVTDANGHIVPDAANRVTFDVKGAGKLVGVDNGSSPDHDSYQADNRKAFSGKVLAIVQSTKEAGEITVTAKADGLQSSTVKIATTAVPGTSTEKTVRSFYYSRNYYVKTGNKPILPSDVEVRYSDGTSDRQNVTWDAVSDDQIAKAGSFSVAGTVAGQKISVRVTMIDEIGAL

SEQ ID NO: 9 - DNA, 3114 bp, Bifidobacterium bifidum
gttgaagatgcaacaagaagcgatagcacaacacaaatgtcatcaacaccggaagttgtttattcatcagcggtcgatagcaaacaaaatcgcacaagcgattttgatgcgaactggaaatttatgctgtcagatagcgttcaagcacaagatccggcatttgatgattcagcatggcaacaagttgatctgccgcatgattatagcatcacacagaaatatagccaaagcaatgaagcagaatcagcatatcttccgggaggcacaggctggtatagaaaaagctttacaattgatagagatctggcaggcaaacgcattgcgattaattttgatggcgtctatatgaatgcaacagtctggtttaatggcgttaaactgggcacacatccgtatggctattcaccgttttcatttgatctgacaggcaatgcaaaatttggcggagaaaacacaattgtcgtcaaagttgaaaatagactgccgtcatcaagatggtattcaggcagcggcatttatagagatgttacactgacagttacagatggcgttcatgttggcaataatggcgtcgcaattaaaacaccgtcactggcaacacaaaatggcggagatgtcacaatgaacctgacaacaaaagtcgcgaatgatacagaagcagcagcgaacattacactgaaacagacagtttttccgaaaggcggaaaaacggatgcagcaattggcacagttacaacagcatcaaaatcaattgcagcaggcgcatcagcagatgttacaagcacaattacagcagcaagcccgaaactgtggtcaattaaaaacccgaacctgtatacagttagaacagaagttctgaacggaggcaaagttctggatacatatgatacagaatatggctttcgctggacaggctttgatgcaacatcaggcttttcactgaatggcgaaaaagtcaaactgaaaggcgttagcatgcatcatgatcaaggctcacttggcgcagttgcaaatagacgcgcaattgaaagacaagtcgaaatcctgcaaaaaatgggcgtcaatagcattcgcacaacacataatccggcagcaaaagcactgattgatgtctgcaatgaaaaaggcgttctggttgtcgaagaagtctttgatatgtggaaccgcagcaaaaatggcaacacggaagattatggcaaatggtttggccaagcaattgcaggcgataatgcagttctgggaggcgataaagatgaaacatgggcgaaatttgatcttacatcaacaattaaccgcgatagaaatgcaccgtcagttattatgtggtcactgggcaatgaaatgatggaaggcatttcaggctcagtttcaggctttccggcaacatcagcaaaactggttgcatggacaaaagcagcagattcaacaagaccgatgacatatggcgataacaaaattaaagcgaactggaacgaatcaaatacaatgggcgataatctgacagcaaatggcggagttgttggcacaaattattcagatggcgcaaactatgataaaattcgtacaacacatccgtcatgggcaatttatggctcagaaacagcatcagcgattaatagccgtggcatttataatagaacaacaggcggagcacaatcatcagataaacagctgacaagctatgataattcagcagttggctggggagcagttgcatcatcagcatggtatgatgttgttcagagagattttgtcgcaggcacatatgtttggacaggatttgattatctgggcgaaccgacaccgtggaatggcacaggctcaggcgcagttggctcatggccgtcaccgaaaaatagctattttggcatcgttgatacagcaggctttccgaaagatacatattatttttatcagagccagtggaatgatgatgttcatacactgcatattcttccggcatggaatgaaaatgttgttgcaaaaggctcaggcaataatgttccggttgtcgtttatacagatgcagcgaaagtgaaactgtattttacaccgaaaggctcaacagaaaaaagactgatcggcgaaaaatcatttacaaaaaaaacaacagcggcaggctatacatatcaagtctatgaaggcagcgataaagattcaacagcgcataaaaacatgtatctgacatggaatgttccgtgggcagaaggcacaatttcagcggaagcgtatgatgaaaataatcgcctgattccggaaggcagcacagaaggcaacgcatcagttacaacaacaggcaaagcagcaaaactgaaagcagatgcggatcgcaaaacaattacagcggatggcaaagatctgtcatatattgaagtcgatgtcacagatgcaaatggccatattgttccggatgcagcaaatagagtcacatttgatgttaaaggcgcaggcaaactggttggcgttgataatggctcatcaccggatcatgattcatatcaagcggataaccgcaaagcattttcaggcaaagtcctggcaattgttcagtcaacaaaagaagcaggcgaaattacagttacagcaaaagcagatggcctgcaatcaagcacagttaaaattgcaacaacagcagttccgggaacaagcacagaaaaaacagtccgcagcttttattacagccgcaactattatgtcaaaacaggcaacaaaccgattctgccgtcagatgttgaagttcgctattcagatggaacaagcgatagacaaaacgttacatgggatgcagtttcagatgatcaaattgcaaaagcaggctcattttcagttgcaggcacagttgcaggccaaaaaattagcgttcgcgtcacaatgattgatgaaattggcgcactgctgaattattcagcaagcacaccggttggcacaccggcagttcttccgggatcaagaccggcagtcctgccggatggcacagtcacatcagcaaattttgcagtccattggacaaaaccggcagatacagtctataatacagcaggcacagtcaaagtaccgggaacagcaacagtttttggcaaagaatttaaagtcacagcgacaattagagttcaa

SEQ ID NO: 10 - protein, 1038 aa, Bifidobacterium bifidum
VEDATRSDSTTQMSSTPEVVYSSAVDSKQNRTSDFDANWKFMLSDSVQAQDPAFDDSAWQQVDLPHDYSITQKYSQSNEAESAYLPGGTGWYRKSFTIDRDLAGKRIAINFDGVYMNATVWFNGVKLGTHPYGYSPFSFDLTGNAKFGGENTIVVKVENRLPSSRWYSGSGIYRDVTLTVTDGVHVGNNGVAIKTPSLATQNGGDVTMNLTTKVANDTEAAANITLKQTVFPKGGKTDAAIGTVTTASKSIAAGASADVTSTITAASPKLWSIKNPNLYTVRTEVLNGGKVLDTYDTEYGFRWTGFDATSGFSLNGEKVKLKGVSMHHDQGSLGAVANRRAIERQVEILQKMGVNSIRTTHNPAAKALIDVCNEKGVLVVEEVFDMWNRSKNGNTEDYGKWFGQAIAGDNAVLGGDKDETWAKFDLTSTINRDRNAPSVIMWSLGNEMMEGISGSVSGFPATSAKLVAWTKAADSTRPMTYGDNKIKANWNESNTMGDNLTANGGVVGTNYSDGANYDKIRTTHPSWAIYGSETASAINSRGIYNRTTGGAQSSDKQLTSYDNSAVGWGAVASSAWYDVVQRDFVAGTYVWTGFDYLGEPTPWNGTGSGAVGSWPSPKNSYFGIVDTAGFPKDTYYFYQSQWNDDVHTLHILPAWNENVVAKGSGNNVPVVVYTDAAKVKLYFTPKGSTEKRLIGEKSFTKKTTAAGYTYQVYEGSDKDSTAHKNMYLTWNVPWAEGTISAEAYDENNRLIPEGSTEGNASVTTTGKAAKLKADADRKTITADGKDLSYIEVDVTDANGHIVPDAANRVTFDVKGAGKLVGVDNGSSPDHDSYQADNRKAFSGKVLAIVQSTKEAGEITVTAKADGLQSSTVKIATTAVPGTSTEKTVRSFYYSRNYYVKTGNKPILPSDVEVRYSDGTSDRQNVTWDAVSDDQIAKAGSFSVAGTVAGQKISVRVTMIDEIGALLNYSASTPVGTPAVLPGSRPAVLPDGTVTSANFAVHWTKPADTVYNTAGTVKVPGTATVFGKEFKVTATIRVQ

SEQ ID NO: 11 - DNA, 3426 bp, Bifidobacterium bifidum
gttgaagatgcaacaagaagcgatagcacaacacaaatgtcatcaacaccggaagttgtttattcatcagcggtcgatagcaaacaaaatcgcacaagcgattttgatgcgaactggaaatttatgctgtcagatagcgttcaagcacaagatccggcatttgatgattcagcatggcaacaagttgatctgccgcatgattatagcatcacacagaaatatagccaaagcaatgaagcagaatcagcatatcttccgggaggcacaggctggtatagaaaaagctttacaattgatagagatctggcaggcaaacgcattgcgattaattttgatggcgtctatatgaatgcaacagtctggtttaatggcgttaaactgggcacacatccgtatggctattcaccgttttcatttgatctgacaggcaatgcaaaatttggcggagaaaacacaattgtcgtcaaagttgaaaatagactgccgtcatcaagatggtattcaggcagcggcatttatagagatgttacactgacagttacagatggcgttcatgttggcaataatggcgtcgcaattaaaacaccgtcactggcaacacaaaatggcggagatgtcacaatgaacctgacaacaaaagtcgcgaatgatacagaagcagcagcgaacattacactgaaacagacagtttttccgaaaggcggaaaaacggatgcagcaattggcacagttacaacagcatcaaaatcaattgcagcaggcgcatcagcagatgttacaagcacaattacagcagcaagcccgaaactgtggtcaattaaaaacccgaacctgtatacagttagaacagaagttctgaacggaggcaaagttctggatacatatgatacagaatatggctttcgctggacaggctttgatgcaacatcaggcttttcactgaatggcgaaaaagtcaaactgaaaggcgttagcatgcatcatgatcaaggctcacttggcgcagttgcaaatagacgcgcaattgaaagacaagtcgaaatcctgcaaaaaatgggcgtcaatagcattcgcacaacacataatccggcagcaaaagcactgattgatgtctgcaatgaaaaaggcgttctggttgtcgaagaagtctttgatatgtggaaccgcagcaaaaatggcaacacggaagattatggcaaatggtttggccaagcaattgcaggcgataatgcagttctgggaggcgataaagatgaaacatgggcgaaatttgatcttacatcaacaattaaccgcgatagaaatgcaccgtcagttattatgtggtcactgggcaatgaaatgatggaaggcatttcaggctcagtttcaggctttccggcaacatcagcaaaactggttgcatggacaaaagcagcagattcaacaagaccgatgacatatggcgataacaaaattaaagcgaactggaacgaatcaaatacaatgggcgataatctgacagcaaatggcggagttgttggcacaaattattcagatggcgcaaactatgataaaattcgtacaacacatccgtcatgggcaatttatggctcagaaacagcatcagcgattaatagccgtggcatttataatagaacaacaggcggagcacaatcatcagataaacagctgacaagctatgataattcagcagttggctggggagcagttgcatcatcagcatggtatgatgttgttcagagagattttgtcgcaggcacatatgtttggacaggatttgattatctgggcgaaccgacaccgtggaatggcacaggctcaggcgcagttggctcatggccgtcaccgaaaaatagctattttggcatcgttgatacagcaggctttccgaaagatacatattatttttatcagagccagtggaatgatgatgttcatacactgcatattcttccggcatggaatgaaaatgttgttgcaaaaggctcaggcaataatgttccggttgtcgtttatacagatgcagcgaaagtgaaactgtattttacaccgaaaggctcaacagaaaaaagactgatcggcgaaaaatcatttacaaaaaaaacaacagcggcaggctatacatatcaagtctatgaaggcagcgataaagattcaacagcgcataaaaacatgtatctgacatggaatgttccgtgggcagaaggcacaatttcagcggaagcgtatgatgaaaataatcgcctgattccggaaggcagcacagaaggcaacgcatcagttacaacaacaggcaaagcagcaaaactgaaagcagatgcggatcgcaaaacaattacagcggatggcaaagatctgtcatatattgaagtcgatgtcacagatgcaaatggccatattgttccggatgcagcaaatagagtcacatttgatgttaaaggcgcaggcaaactggttggcgttgataatggctcatcaccggatcatgattcatatcaagcggataaccgcaaagcattttcaggcaaagtcctggcaattgttcagtcaacaaaagaagcaggcgaaattacagttacagcaaaagcagatggcctgcaatcaagcacagttaaaattgcaacaacagcagttccgggaacaagcacagaaaaaacagtccgcagcttttattacagccgcaactattatgtcaaaacaggcaacaaaccgattctgccgtcagatgttgaagttcgctattcagatggaacaagcgatagacaaaacgttacatgggatgcagtttcagatgatcaaattgcaaaagcaggctcattttcagttgcaggcacagttgcaggccaaaaaattagcgttcgcgtcacaatgattgatgaaattggcgcactgctgaattattcagcaagcacaccggttggcacaccggcagttcttccgggatcaagaccggcagtcctgccggatggcacagtcacatcagcaaattttgcagtccattggacaaaaccggcagatacagtctataatacagcaggcacagtcaaagtaccgggaacagcaacagtttttggcaaagaatttaaagtcacagcgacaattagagttcaaagaagccaagttacaattggctcatcagtttcaggaaatgcactgagactgacacaaaatattccggcagataaacaatcagatacactggatgcgattaaagatggctcaacaacagttgatgcaaatacaggcggaggcgcaaatccgtcagcatggacaaattgggcatattcaaaagcaggccataacacagcggaaattacatttgaatatgcgacagaacaacaactgggccagatcgtcatgtatttttttcgcgatagcaatgcagttagatttccggatgctggcaaaacaaaaattcagatc

SEQ ID NO: 12 - protein, 1142 aa, Bifidobacterium bifidum
VEDATRSDSTTQMSSTPEVVYSSAVDSKQNRTSDFDANWKFMLSDSVQAQDPAFDDSAWQQVDLPHDYSITQKYSQSNEAESAYLPGGTGWYRKSFTIDRDLAGKRIAINFDGVYMNATVWFNGVKLGTHPYGYSPFSFDLTGNAKFGGENTIVVKVENRLPSSRWYSGSGIYRDVTLTVTDGVHVGNNGVAIKTPSLATQNGGDVTMNLTTKVANDTEAAANITLKQTVFPKGGKTDAAIGTVTTASKSIAAGASADVTSTITAASPKLWSIKNPNLYTVRTEVLNGGKVLDTYDTEYGFRWTGFDATSGFSLNGEKVKLKGVSMHHDQGSLGAVANRRAIERQVEILQKMGVNSIRTTHNPAAKALIDVCNEKGVLVVEEVFDMWNRSKNGNTEDYGKWFGQAIAGDNAVLGGDKDETWAKFDLTSTINRDRNAPSVIMWSLGNEMMEGISGSVSGFPATSAKLVAWTKAADSTRPMTYGDNKIKANWNESNTMGDNLTANGGVVGTNYSDGANYDKIRTTHPSWAIYGSETASAINSRGIYNRTTGGAQSSDKQLTSYDNSAVGWGAVASSAWYDVVQRDFVAGTYVWTGFDYLGEPTPWNGTGSGAVGSWPSPKNSYFGIVDTAGFPKDTYYFYQSQWNDDVHTLHILPAWNENVVAKGSGNNVPVVVYTDAAKVKLYFTPKGSTEKRLIGEKSFTKKTTAAGYTYQVYEGSDKDSTAHKNMYLTWNVPWAEGTISAEAYDENNRLIPEGSTEGNASVTTTGKAAKLKADADRKTITADGKDLSYIEVDVTDANGHIVPDAANRVTFDVKGAGKLVGVDNGSSPDHDSYQADNRKAFSGKVLAIVQSTKEAGEITVTAKADGLQSSTVKIATTAVPGTSTEKTVRSFYYSRNYYVKTGNKPILPSDVEVRYSDGTSDRQNVTWDAVSDDQIAKAGSFSVAGTVAGQKISVRVTMIDEIGALLNYSASTPVGTPAVLPGSRPAVLPDGTVTSANFAVHWTKPADTVYNTAGTVKVPGTATVFGKEFKVTATIRVQRSQVTIGSSVSGNALRLTQNIPADKQSDTLDAIKDGSTTVDANTGGGANPSAWTNWAYSKAGHNTAEITFEYATEQQLGQIVMYFFRDSNAVRFPDAGKTKIQI

SEQ ID NO: 13 - DNA, 3633 bp, Bifidobacterium bifidum
gttgaagatgcaacaagaagcgatagcacaacacaaatgtcatcaacaccggaagttgtttattcatcagcggtcgatagcaaacaaaatcgcacaagcgattttgatgcgaactggaaatttatgctgtcagatagcgttcaagcacaagatccggcatttgatgattcagcatggcaacaagttgatctgccgcatgattatagcatcacacagaaatatagccaaagcaatgaagcagaatcagcatatcttccgggaggcacaggctggtatagaaaaagctttacaattgatagagatctggcaggcaaacgcattgcgattaattttgatggcgtctatatgaatgcaacagtctggtttaatggcgttaaactgggcacacatccgtatggctattcaccgttttcatttgatctgacaggcaatgcaaaatttggcggagaaaacacaattgtcgtcaaagttgaaaatagactgccgtcatcaagatggtattcaggcagcggcatttatagagatgttacactgacagttacagatggcgttcatgttggcaataatggcgtcgcaattaaaacaccgtcactggcaacacaaaatggcggagatgtcacaatgaacctgacaacaaaagtcgcgaatgatacagaagcagcagcgaacattacactgaaacagacagtttttccgaaaggcggaaaaacggatgcagcaattggcacagttacaacagcatcaaaatcaattgcagcaggcgcatcagcagatgttacaagcacaattacagcagcaagcccgaaactgtggtcaattaaaaacccgaacctgtatacagttagaacagaagttctgaacggaggcaaagttctggatacatatgatacagaatatggctttcgctggacaggctttgatgcaacatcaggcttttcactgaatggcgaaaaagtcaaactgaaaggcgttagcatgcatcatgatcaaggctcacttggcgcagttgcaaatagacgcgcaattgaaagacaagtcgaaatcctgcaaaaaatgggcgtcaatagcattcgcacaacacataatccggcagcaaaagcactgattgatgtctgcaatgaaaaaggcgttctggttgtcgaagaagtctttgatatgtggaaccgcagcaaaaatggcaacacggaagattatggcaaatggtttggccaagcaattgcaggcgataatgcagttctgggaggcgataaagatgaaacatgggcgaaatttgatcttacatcaacaattaaccgcgatagaaatgcaccgtcagttattatgtggtcactgggcaatgaaatgatggaaggcatttcaggctcagtttcaggctttccggcaacatcagcaaaactggttgcatggacaaaagcagcagattcaacaagaccgatgacatatggcgataacaaaattaaagcgaactggaacgaatcaaatacaatgggcgataatctgacagcaaatggcggagttgttggcacaaattattcagatggcgcaaactatgataaaattcgtacaacacatccgtcatgggcaatttatggctcagaaacagcatcagcgattaatagccgtggcatttataatagaacaacaggcggagcacaatcatcagataaacagctgacaagctatgataattcagcagttggctggggagcagttgcatcatcagcatggtatgatgttgttcagagagattttgtcgcaggcacatatgtttggacaggatttgattatctgggcgaaccgacaccgtggaatggcacaggctcaggcgcagttggctcatggccgtcaccgaaaaatagctattttggcatcgttgatacagcaggctttccgaaagatacatattatttttatcagagccagtggaatgatgatgttcatacactgcatattcttccggcatggaatgaaaatgttgttgcaaaaggctcaggcaataatgttccggttgtcgtttatacagatgcagcgaaagtgaaactgtattttacaccgaaaggctcaacagaaaaaagactgatcggcgaaaaatcatttacaaaaaaaacaacagcggcaggctatacatatcaagtctatgaaggcagcgataaagattcaacagcgcataaaaacatgtatctgacatggaatgttccgtgggcagaaggcacaatttcagcggaagcgtatgatgaaaataatcgcctgattccggaaggcagcacagaaggcaacgcatcagttacaacaacaggcaaagcagcaaaactgaaagcagatgcggatcgcaaaacaattacagcggatggcaaagatctgtcatatattgaagtcgatgtcacagatgcaaatggccatattgttccggatgcagcaaatagagtcacatttgatgttaaaggcgcaggcaaactggttggcgttgataatggctcatcaccggatcatgattcatatcaagcggataaccgcaaagcattttcaggcaaagtcctggcaattgttcagtcaacaaaagaagcaggcgaaattacagttacagcaaaagcagatggcctgcaatcaagcacagttaaaattgcaacaacagcagttccgggaacaagcacagaaaaaacagtccgcagcttttattacagccgcaactattatgtcaaaacaggcaacaaaccgattctgccgtcagatgttgaagttcgctattcagatggaacaagcgatagacaaaacgttacatgggatgcagtttcagatgatcaaattgcaaaagcaggctcattttcagttgcaggcacagttgcaggccaaaaaattagcgttcgcgtcacaatgattgatgaaattggcgcactgctgaattattcagcaagcacaccggttggcacaccggcagttcttccgggatcaagaccggcagtcctgccggatggcacagtcacatcagcaaattttgcagtccattggacaaaaccggcagatacagtctataatacagcaggcacagtcaaagtaccgggaacagcaacagtttttggcaaagaatttaaagtcacagcgacaattagagttcaaagaagccaagttacaattggctcatcagtttcaggaaatgcactgagactgacacaaaatattccggcagataaacaatcagatacactggatgcgattaaagatggctcaacaacagttgatgcaaatacaggcggaggcgcaaatccgtcagcatggacaaattgggcatattcaaaagcaggccataacacagcggaaattacatttgaatatgcgacagaacaacaactgggccagatcgtcatgtatttttttcgcgatagcaatgcagttagatttccggatgctggcaaaacaaaaattcagatcagcgcagatggcaaaaattggacagatctggcagcaacagaaacaattgcagcgcaagaatcaagcgatagagtcaaaccgtatacatatgattttgcaccggttggcgcaacatttgttaaagtgacagtcacaaacgcagatacaacaacaccgtcaggcgttgtttgcgcaggcctgacagaaattgaactgaaaacagcgaca

SEQ ID NO: 14 - protein, 1211 aa, Bifidobacterium bifidum
VEDATRSDSTTQMSSTPEVVYSSAVDSKQNRTSDFDANWKFMLSDSVQAQDPAFDDSAWQQVDLPHDYSITQKYSQSNEAESAYLPGGTGWYRKSFTIDRDLAGKRIAINFDGVYMNATVWFNGVKLGTHPYGYSPFSFDLTGNAKFGGENTIVVKVENRLPSSRWYSGSGIYRDVTLTVTDGVHVGNNGVAIKTPSLATQNGGDVTMNLTTKVANDTEAAANITLKQTVFPKGGKTDAAIGTVTTASKSIAAGASADVTSTITAASPKLWSIKNPNLYTVRTEVLNGGKVLDTYDTEYGFRWTGFDATSGFSLNGEKVKLKGVSMHHDQGSLGAVANRRAIERQVEILQKMGVNSIRTTHNPAAKALIDVCNEKGVLVVEEVFDMWNRSKNGNTEDYGKWFGQAIAGDNAVLGGDKDETWAKFDLTSTINRDRNAPSVIMWSLGNEMMEGISGSVSGFPATSAKLVAWTKAADSTRPMTYGDNKIKANWNESNTMGDNLTANGGVVGTNYSDGANYDKIRTTHPSWAIYGSETASAINSRGIYNRTTGGAQSSDKQLTSYDNSAVGWGAVASSAWYDVVQRDFVAGTYVWTGFDYLGEPTPWNGTGSGAVGSWPSPKNSYFGIVDTAGFPKDTYYFYQSQWNDDVHTLHILPAWNENVVAKGSGNNVPVVVYTDAAKVKLYFTPKGSTEKRLIGEKSFTKKTTAAGYTYQVYEGSDKDSTAHKNMYLTWNVPWAEGTISAEAYDENNRLIPEGSTEGNASVTTTGKAAKLKADADRKTITADGKDLSYIEVDVTDANGHIVPDAANRVTFDVKGAGKLVGVDNGSSPDHDSYQADNRKAFSGKVLAIVQSTKEAGEITVTAKADGLQSSTVKIATTAVPGTSTEKTVRSFYYSRNYYVKTGNKPILPSDVEVRYSDGTSDRQNVTWDAVSDDQIAKAGSFSVAGTVAGQKISVRVTMIDEIGALLNYSASTPVGTPAVLPGSRPAVLPDGTVTSANFAVHWTKPADTVYNTAGTVKVPGTATVFGKEFKVTATIRVQRSQVTIGSSVSGNALRLTQNIPADKQSDTLDAIKDGSTTVDANTGGGANPSAWTNWAYSKAGHNTAEITFEYATEQQLGQIVMYFFRDSNAVRFPDAGKTKIQISADGKNWTDLAATETIAAQESSDRVKPYTYDFAPVGATFVKVTVTNADTTTPSGVVCAGLTEIELKTAT

SEQ ID NO: 15 - DNA, 3888 bp, Bifidobacterium bifidum
gttgaagatgcaacaagaagcgatagcacaacacaaatgtcatcaacaccggaagttgtttattcatcagcggtcgatagcaaacaaaatcgcacaagcgattttgatgcgaactggaaatttatgctgtcagatagcgttcaagcacaagatccggcatttgatgattcagcatggcaacaagttgatctgccgcatgattatagcatcacacagaaatatagccaaagcaatgaagcagaatcagcatatcttccgggaggcacaggctggtatagaaaaagctttacaattgatagagatctggcaggcaaacgcattgcgattaattttgatggcgtctatatgaatgcaacagtctggtttaatggcgttaaactgggcacacatccgtatggctattcaccgttttcatttgatctgacaggcaatgcaaaatttggcggagaaaacacaattgtcgtcaaagttgaaaatagactgccgtcatcaagatggtattcaggcagcggcatttatagagatgttacactgacagttacagatggcgttcatgttggcaataatggcgtcgcaattaaaacaccgtcactggcaacacaaaatggcggagatgtcacaatgaacctgacaacaaaagtcgcgaatgatacagaagcagcagcgaacattacactgaaacagacagtttttccgaaaggcggaaaaacggatgcagcaattggcacagttacaacagcatcaaaatcaattgcagcaggcgcatcagcagatgttacaagcacaattacagcagcaagcccgaaactgtggtcaattaaaaacccgaacctgtatacagttagaacagaagttctgaacggaggcaaagttctggatacatatgatacagaatatggctttcgctggacaggctttgatgcaacatcaggcttttcactgaatggcgaaaaagtcaaactgaaaggcgttagcatgcatcatgatcaaggctcacttggcgcagttgcaaatagacgcgcaattgaaagacaagtcgaaatcctgcaaaaaatgggcgtcaatagcattcgcacaacacataatccggcagcaaaagcactgattgatgtctgcaatgaaaaaggcgttctggttgtcgaagaagtctttgatatgtggaaccgcagcaaaaatggcaacacggaagattatggcaaatggtttggccaagcaattgcaggcgataatgcagttctgggaggcgataaagatgaaacatgggcgaaatttgatcttacatcaacaattaaccgcgatagaaatgcaccgtcagttattatgtggtcactgggcaatgaaatgatggaaggcatttcaggctcagtttcaggctttccggcaacatcagcaaaactggttgcatggacaaaagcagcagattcaacaagaccgatgacatatggcgataacaaaattaaagcgaactggaacgaatcaaatacaatgggcgataatctgacagcaaatggcggagttgttggcacaaattattcagatggcgcaaactatgataaaattcgtacaacacatccgtcatgggcaatttatggctcagaaacagcatcagcgattaatagccgtggcatttataatagaacaacaggcggagcacaatcatcagataaacagctgacaagctatgataattcagcagttggctggggagcagttgcatcatcagcatggtatgatgttgttcagagagattttgtcgcaggcacatatgtttggacaggatttgattatctgggcgaaccgacaccgtggaatggcacaggctcaggcgcagttggctcatggccgtcaccgaaaaatagctattttggcatcgttgatacagcaggctttccgaaagatacatattatttttatcagagccagtggaatgatgatgttcatacactgcatattcttccggcatggaatgaaaatgttgttgcaaaaggctcaggcaataatgttccggttgtcgtttatacagatgcagcgaaagtgaaactgtattttacaccgaaaggctcaacagaaaaaagactgatcggcgaaaaatcatttacaaaaaaaacaacagcggcaggctatacatatcaagtctatgaaggcagcgataaagattcaacagcgcataaaaacatgtatctgacatggaatgttccgtgggcagaaggcacaatttcagcggaagcgtatgatgaaaataatcgcctgattccggaaggcagcacagaaggcaacgcatcagttacaacaacaggcaaagcagcaaaactgaaagcagatgcggatcgcaaaacaattacagcggatggcaaagatctgtcatatattgaagtcgatgtcacagatgcaaatggccatattgttccggatgcagcaaatagagtcacatttgatgttaaaggcgcaggcaaactggttggcgttgataatggctcatcaccggatcatgattcatatcaagcggataaccgcaaagcattttcaggcaaagtcctggcaattgttcagtcaacaaaagaagcaggcgaaattacagttacagcaaaagcagatggcctgcaatcaagcacagttaaaattgcaacaacagcagttccgggaacaagcacagaaaaaacagtccgcagcttttattacagccgcaactattatgtcaaaacaggcaacaaaccgattctgccgtcagatgttgaagttcgctattcagatggaacaagcgatagacaaaacgttacatgggatgcagtttcagatgatcaaattgcaaaagcaggctcattttcagttgcaggcacagttgcaggccaaaaaattagcgttcgcgtcacaatgattgatgaaattggcgcactgctgaattattcagcaagcacaccggttggcacaccggcagttcttccgggatcaagaccggcagtcctgccggatggcacagtcacatcagcaaattttgcagtccattggacaaaaccggcagatacagtctataatacagcaggcacagtcaaagtaccgggaacagcaacagtttttggcaaagaatttaaagtcacagcgacaattagagttcaaagaagccaagttacaattggctcatcagtttcaggaaatgcactgagactgacacaaaatattccggcagataaacaatcagatacactggatgcgattaaagatggctcaacaacagttgatgcaaatacaggcggaggcgcaaatccgtcagcatggacaaattgggcatattcaaaagcaggccataacacagcggaaattacatttgaatatgcgacagaacaacaactgggccagatcgtcatgtatttttttcgcgatagcaatgcagttagatttccggatgctggcaaaacaaaaattcagatcagcgcagatggcaaaaattggacagatctggcagcaacagaaacaattgcagcgcaagaatcaagcgatagagtcaaaccgtatacatatgattttgcaccggttggcgcaacatttgttaaagtgacagtcacaaacgcagatacaacaacaccgtcaggcgttgtttgcgcaggcctgacagaaattgaactgaaaacagcgacaagcaaatttgtcacaaatacatcagcagcactgtcatcacttacagtcaatggcacaaaagtttcagattcagttctggcagcaggctcatataacacaccggcaattatcgcagatgttaaagcggaaggcgaaggcaatgcaagcgttacagtccttccggcacatgataatgttattcgcgtcattacagaaagcgaagatcatgtcacacgcaaaacatttacaatcaacctgggcacagaacaagaattt

SEQ ID NO: 16 - protein, 1296 aa, Bifidobacterium bifidum
VEDATRSDSTTQMSSTPEVVYSSAVDSKQNRTSDFDANWKFMLSDSVQAQDPAFDDSAWQQVDLPHDYSITQKYSQSNEAESAYLPGGTGWYRKSFTIDRDLAGKRIAINFDGVYMNATVWFNGVKLGTHPYGYSPFSFDLTGNAKFGGENTIVVKVENRLPSSRWYSGSGIYRDVTLTVTDGVHVGNNGVAIKTPSLATQNGGDVTMNLTTKVANDTEAAANITLKQTVFPKGGKTDAAIGTVTTASKSIAAGASADVTSTITAASPKLWSIKNPNLYTVRTEVLNGGKVLDTYDTEYGFRWTGFDATSGFSLNGEKVKLKGVSMHHDQGSLGAVANRRAIERQVEILQKMGVNSIRTTHNPAAKALIDVCNEKGVLVVEEVFDMWNRSKNGNTEDYGKWFGQAIAGDNAVLGGDKDETWAKFDLTSTINRDRNAPSVIMWSLGNEMMEGISGSVSGFPATSAKLVAWTKAADSTRPMTYGDNKIKANWNESNTMGDNLTANGGVVGTNYSDGANYDKIRTTHPSWAIYGSETASAINSRGIYNRTTGGAQSSDKQLTSYDNSAVGWGAVASSAWYDVVQRDFVAGTYVWTGFDYLGEPTPWNGTGSGAVGSWPSPKNSYFGIVDTAGFPKDTYYFYQSQWNDDVHTLHILPAWNENVVAKGSGNNVPVVVYTDAAKVKLYFTPKGSTEKRLIGEKSFTKKTTAAGYTYQVYEGSDKDSTAHKNMYLTWNVPWAEGTISAEAYDENNRLIPEGSTEGNASVTTTGKAAKLKADADRKTITADGKDLSYIEVDVTDANGHIVPDAANRVTFDVKGAGKLVGVDNGSSPDHDSYQADNRKAFSGKVLAIVQSTKEAGEITVTAKADGLQSSTVKIATTAVPGTSTEKTVRSFYYSRNYYVKTGNKPILPSDVEVRYSDGTSDRQNVTWDAVSDDQIAKAGSFSVAGTVAGQKISVRVTMIDEIGALLNYSASTPVGTPAVLPGSRPAVLPDGTVTSANFAVHWTKPADTVYNTAGTVKVPGTATVFGKEFKVTATIRVQRSQVTIGSSVSGNALRLTQNIPADKQSDTLDAIKDGSTTVDANTGGGANPSAWTNWAYSKAGHNTAEITFEYATEQQLGQIVMYFFRDSNAVRFPDAGKTKIQISADGKNWTDLAATETIAAQESSDRVKPYTYDFAPVGATFVKVTVTNADTTTPSGVVCAGLTEIELKTATSKFVTNTSAALSSLTVNGTKVSDSVLAAGSYNTPAIIADVKAEGEGNASVTVLPAHDNVIRVITESEDHVTRKTFTINLGTEQEF

SEQ ID NO: 17 - protein, 1025 aa, Kluyveromyces lactis
MSCLIPENLRNPKKVHENRLPTRAYYYDQDIFESLNGPWAFALFDAPLDAPDAKNLDWETAKKWSTISVPSHWELQEDWKYGKPIYTNVQYPIPIDIPNPPTVNPTGVYARTFELDSKSIESFEHRLRFEGVDNCYELYVNGQYVGFNKGSRNGAEFDIQKYVSEGENLVVVKVFKWSDSTYIEDQDQWWLSGIYRDVSLLKLPKKAHIEDVRVTTTFVDSQYQDAELSVKVDVQGSSYDHINFTLYEPEDGSKVYDASSLLNEENGNTTFSTKEFISFSTKKNEETAFKINVKAPEHWTAENPTLYKYQLDLIGSDGSVIQSIKHHVGFRQVELKDGNITVNGKDILFRGVNRHDHHPRFGRAVPLDFVVRDLILMKKFNINAVRNSHYPNHPKVYDLFDKLGFWVIDEADLETHGVQEPFNRHTNLEAEYPDTKNKLYDVNAHYLSDNPEYEVAYLDRASQLVLRDVNHPSIIIWSLGNEACYGRNHKAMYKLIKQLDPTRLVHYEGDLNALSADIFSFMYPTFEIMERWRKNHTDENGKFEKPLILCEYGHAMGNGPGSLKEYQELFYKEKFYQGGFIWEWANHGIEFEDVSTADGKLHKAYAYGGDFKEEVHDGVFIMDGLCNSEHNPTPGLVEYKKVIEPVHIKIAHGSVTITNKHDFITTDHLLFIDKDTGKTIDVPSLKPEESVTIPSDTTYVVAVLKDDAGVLKAGHEIAWGQAELPLKVPDFVTETAEKAAKINDGKRYVSVESSGLHFILDKLLGKIESLKVKGKEISSKFEGSSITFWRPPTNNDEPRDFKNWKKYNIDLMKQNIHGVSVEKGSNGSLAVVTVNSRISPVVFYYGFETVQKYTIFANKINLNTSMKLTGEYQPPDFPRVGYEFWLGDSYESFEWLGRGPGESYPDKKESQRFGLYDSKDVEEFVYDYPQENGNHTDTHFLNIKFEGAGKLSIFQKEKPFNFKISDEYGVDEAAHACDVKRYGRHYLRLDHAIHGVGSEACGPAVLDQYRLKAQDFNFEFDLAFE

SEQ ID NO: 18 - protein, 902 aa, Aspergillus oryzae
SIKHRLNGFTILEHPDPAKRDLLQDIVTWDDKSLFINGERIMLFSGEVHPFRLPVPSLWLDIFHKIRALGFNCVSFYIDWALLEGKPGDYRAEGIFALEPFFDAAKEAGIYLIARPGSYINAEVSGGGFPGWLQRVNGTLRSSDEPFLKATDNYIANAAAAVAKAQITNGGPVILYQPENEYSGGCCGVKYTDADYMQYVMDQARKADIVVPFISNDASPSGHNAPGSGTGAVDIYGHDSYPLGFDCANPSVWPEGKLPDNFRTLHLEQSPSTPYSLLEFQAGAFDPWGGPGFEKCYALVNHEFSRVFYRNDLSFGVSTFNLYMTFGGTNWGNLGHPGGYTSYDYGSPITETRNVTREKYSDIKLLANFVKASPSYLTATPRNLTTGVYTDTSDLAVTPLIGDSPGSFFVVRHTDYSSQESTSYKLKLPTSAGNLTIPQLEGTLSLNGRDSKIHVVDYNVSGTNIIYSTAEVFTWKKFDGNKVLVLYGGPKEHHELAIASKSNVTIIEGSDSGIVSTRKGSSVIIGWDVSSTRRIVQVGDLRVFLLDRNSAYNYWVPELPTEGTSPGFSTSKTTASSIIVKAGYLLRGAHLDGADLHLTADFNATTPIEVIGAPTGAKNLFVNGEKASHTVDKNGIWSSEVKYAAPEIKLPGLKDLDWKYLDTLPEIKSSYDDSAWVSADLPKTKNTHRPLDTPTSLYSSDYGFHTGYLIYRGHFVANGKESEFFIRTQGGSAFGSSVWLNETYLGSWTGADYAMDGNSTYKLSQLESGKNYVITVVIDNLGLDENWTVGEETMKNPRGILSYKLSGQDASAITWKLTGNLGGEDYQDKVRGPLNEGGLYAERQGFHQPQPPSESWESGSPLEGLSKPGIGFYTAQFDLDLPKGWDVPLYFNFGNNTQAARA

SEQ ID NO: 19 - DNA, 24 bp, Artificial Sequence
  I-SceI-1 oligo
cgattagggataacagggtaatat

SEQ ID NO: 20 - DNA, 24 bp, Artificial Sequence
  I-SceI-2 olio
cgatattaccctgttatccctaat

SEQ ID NO: 21 - DNA, 32 bp, Artificial Sequence
  primer 981
aaccagcactagtgtcgacgcctggtaggtcg

SEQ ID NO: 22 - DNA, 54 bp, Artificial Sequence
  primer 984
gcaccaatgtatcctgttttccccatatcgttagccctttaaccgatcatcatc

SEQ ID NO: 23 - DNA, 37 bp, Artificial Sequence
  primer 985
atatggatccgttctactagacatttatgaagtacag

SEQ ID NO: 24 - DNA, 42 bp, Artificial Sequence
  primer 983
gatgatgatcggttaaagggctaacgatatggggaaaacagg

SEQ ID NO: 25 - DNA, 3027 bp, Lactobacillus delbrueckii
atgagcaataagttagtaaaagaaaaaagagttgaccaggcagacctggcctggctgactgacccggaagtttacgaagtcaatacaattcccccgcactccgaccatgagtccttccaaagccaggaagaactggaggagggcaagtccagtttagtgcagtccctggacggggactggctgattgactacgctgaaaacggccagggaccagtcaacttctatgcagaagactttgacgatagcaattttaagtcagtcaaagtacccggcaacctggaactgcaaggctttggccagccccagtatgtcaacgtccaatatccatgggacggcagtgaggagattttcccgccccaaattccaagcaaaaatccgctcgcttcttatgtcagatactttgacctggatgaagctttctgggacaaggaagtcagcttgaagtttgacggggcggcaacagccatctatgtctggctgaacggccacttcgtcggctacggggaagactcctttaccccaagtgagtttatggttaccaagttcctcaagaaagaaaataaccgcctggcagtggctctctacaagtattcttccgcctcctggctggaagaccaggacttctggcgcatgtctggtttgttcagatcagtgactcttcaggccaagccgcgtctgcacttggaggaccttaagcttacggccagcttgaccgataactaccaaaaaggaaagctggaagtcgaagccaatattgcctaccgcttgccaaatgccagctttaagctggaagtgcgggatagtgaaggtgacttggttgctgaaaagctgggcccaatcagaagcgagcagctggaattcactctggctgatttgccagtagctgcctggagcgcggaaaagcctaacctttaccaggtccgcctgtatttataccaggcaggcagcctcttagaggttagccggcaggaagtgggtttccgcaactttgaactaaaagacgggattatgtaccttaacggccagcggatcgtcttcaagggggccaaccggcacgaatttgacagtaagttgggtcgggctatcacggaagaggatatgatctgggacatcaagaccatgaagcgaagcaacatcaatgctgtccgctgctctcactacccgaaccagtccctcttttaccggctctgtgacaagtacggcctttacgtcattgatgaagctaacctggaaagccacggcacctgggaaaaagtgggggggcacgaagatcctagcttcaatgttccaggcgatgaccagcattggctgggagccagcttatcccgggtgaagaacatgatggctcgggacaagaaccatgcttcaatcctaatctggtctttaggcaatgagtcttacgccggcactgtctttgcccaaatggctgattacgtccggaaggctgatccgacccgggttcagcactatgaaggggtgacccataaccggaagtttgacgacgccacccagattgaaagccggatgtatgctccggccaaggtaattgaagaatacttgaccaataaaccagccaagccatttatctcagttgaatacgctcacgccatgggcaactccgtcggtgacctggccgcctacacggccctggaaaaatacccccactaccagggcggcttcatctgggactggattgaccaaggactggaaaaagacgggcacctgctttatgggggcgacttcgatgaccggccaaccgactatgaattctgcgggaacggcctggtctttgctgaccggactgaatcgccgaaactggctaatgtcaaggccctttacgccaaccttaagttagaagtaaaagatgggcagctcttcctcaaaaacgacaatttatttaccaacagctcatcttactacttcttgactagtcttttggtcgatggcaagttgacctaccagagccggcctctgacctttggcctggagcctggcgaatccgggacctttgccctgccttggccggaagtcgctgatgaaaaaggagaggtcgtctaccgggtaacggcccacttaaaagaagacttgccttgggcggatgagggcttcactgtggctgaagcagaagaagtagctcaaaagctgccggaatttaagccggaagggcggccagatttagttgattccgactacaacctaggcctgaaaggaaataacttccaaattctcttctccaaggtcaagggctggccggtttccctcaagtatgccggtagggaatacttgaagcggctgccggaatttaccttctggcgggccctgacggacaacgaccggggagctggttacggctatgatctggcccggtgggaaaatgccggcaagtatgcccgcttgaaagacatcagctgcgaggtcaaggaagactccgttttggtcaagactgcctttacgttgcctgtcgccttaaagggtgatttaaccgtgacctatgaagtcgatggacggggcaagattgctgtaacagctgacttcccaggcgcggaagaagccggtctcttgccagcctttggcttgaacctggccctgccaaaagaactgaccgattaccgctactatggtctgggacctaatgagagctacccagaccgcttggaaggtaattacctgggcatctaccagggagcggtaaaaaagaactttagcccatacctgcgtccgcaggaaacgggcaaccggagcaaggttcgctggtaccagctctttgatgaaaagggcggcttggaatttacggccaatggggcagacttgaacttgtctgctttgccatattctgccgcccaaattgaagcagcggaccacgcttttgaactgactaacaattacacttgggttagagccttaagcgcccagatgggggtcggcggggatgactcctgggggcagaaggtccacccggaattctgcctggatgctcaaaaagcccgccagctccgcctggtgattcagccccttttactaaaataa

SEQ ID NO: 26 - protein, 1008 aa, Lactobacillus delbrueckii
MSNKLVKEKRVDQADLAWLTDPEVYEVNTIPPHSDHESFQSQEELEEGKSSLVQSLDGDWLIDYAENGQGPVNFYAEDFDDSNFKSVKVPGNLELQGFGQPQYVNVQYPWDGSEEIFPPQIPSKNPLASYVRYFDLDEAFWDKEVSLKFDGAATAIYVWLNGHFVGYGEDSFTPSEFMVTKFLKKENNRLAVALYKYSSASWLEDQDFWRMSGLFRSVTLQAKPRLHLEDLKLTASLTDNYQKGKLEVEANIAYRLPNASFKLEVRDSEGDLVAEKLGPIRSEQLEFTLADLPVAAWSAEKPNLYQVRLYLYQAGSLLEVSRQEVGFRNFELKDGIMYLNGQRIVFKGANRHEFDSKLGRAITEEDMIWDIKTMKRSNINAVRCSHYPNQSLFYRLCDKYGLYVIDEANLESHGTWEKVGGHEDPSFNVPGDDQHWLGASLSRVKNMMARDKNHASILIWSLGNESYAGTVFAQMADYVRKADPTRVQHYEGVTHNRKFDDATQIESRMYAPAKVIEEYLTNKPAKPFISVEYAHAMGNSVGDLAAYTALEKYPHYQGGFIWDWIDQGLEKDGHLLYGGDFDDRPTDYEFCGNGLVFADRTESPKLANVKALYANLKLEVKDGQLFLKNDNLFTNSSSYYFLTSLLVDGKLTYQSRPLTFGLEPGESGTFALPWPEVADEKGEVVYRVTAHLKEDLPWADEGFTVAEAEEVAQKLPEFKPEGRPDLVDSDYNLGLKGNNFQILFSKVKGWPVSLKYAGREYLKRLPEFTFWRALTDNDRGAGYGYDLARWENAGKYARLKDISCEVKEDSVLVKTAFTLPVALKGDLTVTYEVDGRGKIAVTADFPGAEEAGLLPAFGLNLALPKELTDYRYYGLGPNESYPDRLEGNYLGIYQGAVKKNFSPYLRPQETGNRSKVRWYQLFDEKGGLEFTANGADLNLSALPYSAAQIEAADHAFELTNNYTWVRALSAQMGVGGDDSWGQKVHPEFCLDAQKARQLRLVIQPLLLK